European Patent Application EP 4 541 899 A1, published April 23, 2025. Title: A method for producing high-titer virus vector. Applicant: Nippon Medical School Foundation. The sequence listing filed with the application follows.

SEQUENCE LISTING (2 sequences)

SEQ ID NO: 1 - DNA, 20 bp, synthetic construct
  misc_feature 1..20: note = Primer
  source 1..20: mol_type = other DNA
tgaccgagaaggagatcgtg

SEQ ID NO: 2 - DNA, 20 bp, synthetic construct
  misc_feature 1..20: note = Primer
  source 1..20: mol_type = other DNA
gagaatctcgcggatcttgc